European Patent Specification EP 3 747 898 B1, published March 15, 2023. Title: USE OF ICOS-BASED CARS TO ENHANCE ANTITUMOR ACTIVITY AND CAR PERSISTENCE. Applicant: The Trustees of the University of Pennsylvania. Application not yet assigned. The sequence listing filed with the application follows.

SEQUENCE LISTING (16 sequences)

SEQ ID NO: 1 - DNA, 1184 bp, Artificial Sequence
  Chemically Synthesized
cgtgaggctccggtgcccgtcagtgggcagagcgcacatcgcccacagtccccgagaagttggggggaggggtcggcaattgaaccggtgcctagagaaggtggcgcggggtaaactgggaaagtgatgtcgtgtactggctccgcctttttcccgagggtgggggagaaccgtatataagtgcagtagtcgccgtgaacgttctttttcgcaacgggtttgccgccagaacacaggtaagtgccgtgtgtggttcccgcgggcctggcctctttacgggttatggcccttgcgtgccttgaattacttccacctggctgcagtacgtgattcttgatcccgagcttcgggttggaagtgggtgggagagttcgaggccttgcgcttaaggagccccttcgcctcgtgcttgagttgaggcctggcctgggcgctggggccgccgcgtgcgaatctggtggcaccttcgcgcctgtctcgctgctttcgataagtctctagccatttaaaatttttgatgacctgctgcgacgctttttttctggcaagatagtcttgtaaatgcgggccaagatctgcacactggtatttcggtttttggggccgcgggcggcgacggggcccgtgcgtcccagcgcacatgttcggcgaggcggggcctgcgagcgcggccaccgagaatcggacgggggtagtctcaagctggccggcctgctctggtgcctggcctcgcgccgccgtgtatcgccccgccctgggcggcaaggctggcccggtcggcaccagttgcgtgagcggaaagatggccgcttcccggccctgctgcagggagctcaaaatggaggacgcggcgctcgggagagcgggcgggtgagtcacccacacaaaggaaaagggcctttccgtcctcagccgtcgcttcatgtgactccacggagtaccgggcgccgtccaggcacctcgattagttctcgagcttttggagtacgtcgtctttaggttggggggaggggttttatgcgatggagtttccccacactgagtgggtggagactgaagttaggccagcttggcacttgatgtaattctccttggaatttgccctttttgagtttggatcttggttcattctcaagcctcagacagtggttcaaagtttttttcttccatttcaggtgtcgtga

SEQ ID NO: 2 - DNA, 63 bp, Artificial Sequence
  Chemically Synthesized
atggccttaccagtgaccgccttgctcctgccgctggccttgctgctccacgccgccaggccg

SEQ ID NO: 3 - DNA, 720 bp, Artificial Sequence
  Chemically Synthesized
caggtacaactgcagcagtctgggcctgagctggagaagcctggcgcttcagtgaagatatcctgcaaggcttctggttactcattcactggctacaccatgaactgggtgaagcagagccatggaaagagccttgagtggattggacttattactccttacaatggtgcttctagctacaaccagaagttcaggggcaaggccacattaactgtagacaagtcatccagcacagcctacatggacctcctcagtctgacatctgaagactctgcagtctatttctgtgcaagggggggttacgacgggaggggttttgactactggggccaagggaccacggtcaccgtctcctcaggtggaggcggttcaggcggcggtggctctagcggtggcggatcggacatcgagctcactcagtctccagcaatcatgtctgcatctccaggggagaaggtcaccatgacctgcagtgccagctcaagtgtaagttacatgcactggtaccagcagaagtcaggcacctcccccaaaagatggatttatgacacatccaaactggcttctggagtcccaggtcgcttcagtggcagtgggtctggaaactcttactctctcacaatcagcagcgtggaggctgaagatgatgcaacttattactgccagcagtggagtaagcaccctctcacgtacggtgctgggacaaagttggaaatcaaa

SEQ ID NO: 4 - DNA, 135 bp, Artificial Sequence
  Chemically Synthesized
accacgacgccagcgccgcgaccaccaacaccggcgcccaccatcgcgtcgcagcccctgtccctgcgcccagaggcgtgccggccagcggcggggggcgcagtgcacacgagggggctggacttcgcctgtgat

SEQ ID NO: 5 - DNA, 72 bp, Artificial Sequence
  Chemically Synthesized
ttctggttacccataggatgtgcagcctttgttgtagtctgcattttgggatgcatacttatttgttggctt

SEQ ID NO: 6 - DNA, 105 bp, Artificial Sequence
  Chemically Synthesized
acaaaaaagaagtattcatccagtgtgcacgaccctaacggtgaatacatgttcatgagagcagtgaacacagccaaaaaatccagactcacagatgtgacccta

SEQ ID NO: 7 - DNA, 336 bp, Artificial Sequence
  Chemically Synthesized
agagtgaagttcagcaggagcgcagacgcccccgcgtacaagcagggccagaaccagctctataacgagctcaatctaggacgaagagaggagtacgatgttttggacaagagacgtggccgggaccctgagatggggggaaagccgagaaggaagaaccctcaggaaggcctgtacaatgaactgcagaaagataagatggcggaggcctacagtgagattgggatgaaaggcgagcgccggaggggcaaggggcacgatggcctttaccagggtctcagtacagccaccaaggacacctacgacgcccttcacatgcaggccctgccccctcgc

SEQ ID NO: 8 - DNA, 1455 bp, Artificial Sequence
  Chemically Synthesized
atggccttaccagtgaccgccttgctcctgccgctggccttgctgctccacgccgccaggccgggatcccaggtacaactgcagcagtctgggcctgagctggagaagcctggcgcttcagtgaagatatcctgcaaggcttctggttactcattcactggctacaccatgaactgggtgaagcagagccatggaaagagccttgagtggattggacttattactccttacaatggtgcttctagctacaaccagaagttcaggggcaaggccacattaactgtagacaagtcatccagcacagcctacatggacctcctcagtctgacatctgaagactctgcagtctatttctgtgcaagggggggttacgacgggaggggttttgactactggggccaagggaccacggtcaccgtctcctcaggtggaggcggttcaggcggcggtggctctagcggtggcggatcggacatcgagctcactcagtctccagcaatcatgtctgcatctccaggggagaaggtcaccatgacctgcagtgccagctcaagtgtaagttacatgcactggtaccagcagaagtcaggcacctcccccaaaagatggatttatgacacatccaaactggcttctggagtcccaggtcgcttcagtggcagtgggtctggaaactcttactctctcacaatcagcagcgtggaggctgaagatgatgcaacttattactgccagcagtggagtaagcaccctctcacgtacggtgctgggacaaagttggaaatcaaagctagcaccacgacgccagcgccgcgaccaccaacaccggcgcccaccatcgcgtcgcagcccctgtccctgcgcccagaggcgtgccggccagcggcggggggcgcagtgcacacgagggggctggacttcgcctgtgatttcgaattctggttacccataggatgtgcagcctttgttgtagtctgcattttgggatgcatacttatttgttggcttacaaaaaagaagtattcatccagtgtgcacgaccctaacggtgaatacatgttcatgagagcagtgaacacagccaaaaaatccagactcacagatgtgaccctaactagtagagtgaagttcagcaggagcgcagacgcccccgcgtacaagcagggccagaaccagctctataacgagctcaatctaggacgaagagaggagtacgatgttttggacaagagacgtggccgggaccctgagatggggggaaagccgagaaggaagaaccctcaggaaggcctgtacaatgaactgcagaaagataagatggcggaggcctacagtgagattgggatgaaaggcgagcgccggaggggcaaggggcacgatggcctttaccagggtctcagtacagccaccaaggacacctacgacgcccttcacatgcaggccctgccccctcgc

SEQ ID NO: 9 - protein, 21 aa, Artificial Sequence
  Chemically Synthesized
MALPVTALLLPLALLLHAARP

SEQ ID NO: 10 - protein, 240 aa, Artificial Sequence
  Chemically Synthesized
QVQLQQSGPELEKPGASVKISCKASGYSFTGYTMNWVKQSHGKSLEWIGLITPYNGASSYNQKFRGKATLTVDKSSSTAYMDLLSLTSEDSAVYFCARGGYDGRGFDYWGQGTTVTVSSGGGGSGGGGSSGGGSDIELTQSPAIMSASPGEKVTMTCSASSSVSYMHWYQQKSGTSPKRWIYDTSKLASGVPGRFSGSGSGNSYSLTISSVEAEDDATYYCQQWSKHPLTYGAGTKLEIK

SEQ ID NO: 11 - protein, 45 aa, Artificial Sequence
  Chemically Synthesized
TTTPAPRPPTPAPTIASQPLSLRPEACRPAAGGAVHTRGLDFACD

SEQ ID NO: 12 - protein, 24 aa, Artificial Sequence
  Chemically Synthesized
FWLPIGCAAFVVVCILGCILICWL

SEQ ID NO: 13 - protein, 35 aa, Artificial Sequence
  Chemically Synthesized
TKKKYSSSVHDPNGEYMFMRAVNTAKKSRLTDVTL

SEQ ID NO: 14 - protein, 112 aa, Artificial Sequence
  Chemically Synthesized
RVKFSRSADAPAYKQGQNQLYNELNLGRREEYDVLDKRRGRDPEMGGKPRRKNPQEGLYNELQKDKMAEAYSEIGMKGERRRGKGHDGLYQGLSTATKDTYDALHMQALPPR

SEQ ID NO: 15 - protein, 485 aa, Artificial Sequence
  Chemically Synthesized
MALPVTALLLPLALLLHAARPGSQVQLQQSGPELEKPGASVKISCKASGYSFTGYTMNWVKQSHGKSLEWIGLITPYNGASSYNQKFRGKATLTVDKSSSTAYMDLLSLTSEDSAVYFCARGGYDGRGFDYWGQGTTVTVSSGGGGSGGGGSSGGGSDIELTQSPAIMSASPGEKVTMTCSASSSVSYMHWYQQKSGTSPKRWIYDTSKLASGVPGRFSGSGSGNSYSLTISSVEAEDDATYYCQQWSKHPLTYGAGTKLEIKASTTTPAPRPPTPAPTIASQPLSLRPEACRPAAGGAVHTRGLDFACDFEFWLPIGCAAFVVVCILGCILICWLTKKKYSSSVHDPNGEYMFMRAVNTAKKSRLTDVTLTSRVKFSRSADAPAYKQGQNQLYNELNLGRREEYDVLDKRRGRDPEMGGKPRRKNPQEGLYNELQKDKMAEAYSEIGMKGERRRGKGHDGLYQGLSTATKDTYDALHMQALPPR

SEQ ID NO: 16 - DNA, 2651 bp, Artificial Sequence
  Chemically Synthesized
cgtgaggctccggtgcccgtcagtgggcagagcgcacatcgcccacagtccccgagaagttggggggaggggtcggcaattgaaccggtgcctagagaaggtggcgcggggtaaactgggaaagtgatgtcgtgtactggctccgcctttttcccgagggtgggggagaaccgtatataagtgcagtagtcgccgtgaacgttctttttcgcaacgggtttgccgccagaacacaggtaagtgccgtgtgtggttcccgcgggcctggcctctttacgggttatggcccttgcgtgccttgaattacttccacctggctgcagtacgtgattcttgatcccgagcttcgggttggaagtgggtgggagagttcgaggccttgcgcttaaggagccccttcgcctcgtgcttgagttgaggcctggcctgggcgctggggccgccgcgtgcgaatctggtggcaccttcgcgcctgtctcgctgctttcgataagtctctagccatttaaaatttttgatgacctgctgcgacgctttttttctggcaagatagtcttgtaaatgcgggccaagatctgcacactggtatttcggtttttggggccgcgggcggcgacggggcccgtgcgtcccagcgcacatgttcggcgaggcggggcctgcgagcgcggccaccgagaatcggacgggggtagtctcaagctggccggcctgctctggtgcctggcctcgcgccgccgtgtatcgccccgccctgggcggcaaggctggcccggtcggcaccagttgcgtgagcggaaagatggccgcttcccggccctgctgcagggagctcaaaatggaggacgcggcgctcgggagagcgggcgggtgagtcacccacacaaaggaaaagggcctttccgtcctcagccgtcgcttcatgtgactccacggagtaccgggcgccgtccaggcacctcgattagttctcgtgcttttggagtacgtcgtctttaggttggggggaggggttttatgcgatggagtttccccacactgagtgggtggagactgaagttaggccagcttggcacttgatgtaattctccttggaatttgccctttttgagtttggatcttggttcattctcaagcctcagacagtggttcaaagtttttttcttccatttcaggtgtcgtgagctagctctagaatggccttaccagtgaccgccttgctcctgccgctggccttgctgctccacgccgccaggccgggatcccaggtacaactgcagcagtctgggcctgagctggagaagcctggcgcttcagtgaagatatcctgcaaggcttctggttactcattcactggctacaccatgaactgggtgaagcagagccatggaaagagccttgagtggattggacttattactccttacaatggtgcttctagctacaaccagaagttcaggggcaaggccacattaactgtagacaagtcatccagcacagcctacatggacctcctcagtctgacatctgaagactctgcagtctatttctgtgcaagggggggttacgacgggaggggttttgactactggggccaagggaccacggtcaccgtctcctcaggtggaggcggttcaggcggcggtggctctagcggtggcggatcggacatcgagctcactcagtctccagcaatcatgtctgcatctccaggggagaaggtcaccatgacctgcagtgccagctcaagtgtaagttacatgcactggtaccagcagaagtcaggcacctcccccaaaagatggatttatgacacatccaaactggcttctggagtcccaggtcgcttcagtggcagtgggtctggaaactcttactctctcacaatcagcagcgtggaggctgaagatgatgcaacttattactgccagcagtggagtaagcaccctctcacgtacggtgctgggacaaagttggaaatcaaagctagcaccacgacgccagcgccgcgaccaccaacaccggcgcccaccatcgcgtcgcagcccctgtccctgcgcccagaggcgtgccggccagcggcggggggcgcagtgcacacgagggggctggacttcgcctgtgatttcgaattctggttacccataggatgtgcagcctttgttgtagtctgcattttgggatgcatacttatttgttggcttacaaaaaagaagtattcatccagtgtgcacgaccctaacggtgaatacatgttcatgagagcagtgaacacagccaaaaaatccagactcacagatgtgaccctaactagtagagtgaagttcagcaggagcgcagacgcccccgcgtacaagcagggccagaaccagctctataacgagctcaatctaggacgaagagaggagtacgatgttttggacaagagacgtggccgggaccctgagatggggggaaagccgagaaggaagaaccctcaggaaggcctgtacaatgaactgcagaaagataagatggcggaggcctacagtgagattgggatgaaaggcgagcgccggaggggcaaggggcacgatggcctttaccagggtctcagtacagccaccaaggacacctacgacgcccttcacatgcaggccctgccccctcgc